European Patent Application EP 4 745 150 A1, published May 20, 2026. Title: Composition for strengthening eyebrow or eyelash. Applicant: AMOREPACIFIC CORPORATION. The sequence listing filed with the application follows.

SEQUENCE LISTING (22 sequences)

SEQ ID NO: 1 - protein, 6 aa, synthetic construct
CKFCKF

SEQ ID NO: 2 - protein, 9 aa, synthetic construct
CKFCKFCKF

SEQ ID NO: 3 - protein, 12 aa, synthetic construct
CKFCKFCKFCKF

SEQ ID NO: 4 - protein, 6 aa, synthetic construct
CWKCWK

SEQ ID NO: 5 - protein, 9 aa, synthetic construct
CWKCWKCWK

SEQ ID NO: 6 - protein, 12 aa, synthetic construct
CWKCWKCWKCWK

SEQ ID NO: 7 - protein, 6 aa, synthetic construct
KCVKCV

SEQ ID NO: 8 - protein, 9 aa, synthetic construct
KCVKCVKCV

SEQ ID NO: 9 - protein, 12 aa, synthetic construct
KCVKCVKCVKCV

SEQ ID NO: 10 - protein, 11 aa, synthetic construct
CCQSSCCKPSC

SEQ ID NO: 11 - protein, 11 aa, synthetic construct
CVSSCCKPQCC

SEQ ID NO: 12 - protein, 10 aa, synthetic construct
PIYCRRTCYH

SEQ ID NO: 13 - protein, 10 aa, synthetic construct
DCKLPCNPCA

SEQ ID NO: 14 - protein, 10 aa, synthetic construct
CLPCLPAASC

SEQ ID NO: 15 - protein, 10 aa, synthetic construct
CEPAICEPSC

SEQ ID NO: 16 - protein, 11 aa, synthetic construct
CQCSCCKPYCS

SEQ ID NO: 17 - protein, 13 aa, synthetic construct
GGVCGPSPPCITT

SEQ ID NO: 18 - protein, 15 aa, synthetic construct
CWKCWKKCLKCLKCV

SEQ ID NO: 19 - protein, 15 aa, synthetic construct
CKWCWKKCLKCVKCL

SEQ ID NO: 20 - protein, 15 aa, synthetic construct
CKWKCFCKFCWKKCV

SEQ ID NO: 21 - protein, 15 aa, synthetic construct
KCFKCFCKWCKFKCV

SEQ ID NO: 22 - protein, 15 aa, synthetic construct
CKFCKWKCFKCVKCF